European Patent Application EP 4 737 480 A1, published May 6, 2026. Title: ＨＥＲ２分解活性を有する抗体軽鎖由来のポリペプチド、前記ポリペプチドを含むＨＥＲ２結合ポリペプチド、これらの製造法及びこれらの用途. Applicant: 国立研究開発法人科学技術振興機構. The sequence listing filed with the application follows.

SEQUENCE LISTING (15 sequences)

SEQ ID NO: 1 - protein, 11 aa, synthetic construct
RASQDVNTAVA

SEQ ID NO: 2 - protein, 7 aa, synthetic construct
SASFLYS

SEQ ID NO: 3 - protein, 9 aa, synthetic construct
QQHYTTPPT

SEQ ID NO: 4 - protein, 214 aa, synthetic construct
DIQMTQSPSSLSASVGDRVTITCRASQDVNTAVAWYQQKPGKAPKLLIYSASFLYSGVPSRFSGSRSGTDFTLTISSLQPEDFATYYCQQHYTTPPTFGQGTKVEIKRTVAAPSVFIFPPSDEQLKSGTASVVCLLNNFYPREAKVQWKVDNALQSGNSQESVTEQDSKDSTYSLSSTLTLSKADYEKHKVYACEVTHQGLSSPVTKSFNRGEC

SEQ ID NO: 5 - protein, 7 aa, synthetic construct
QQHYTTT

SEQ ID NO: 6 - protein, 212 aa, synthetic construct
DIQMTQSPSSLSASVGDRVTITCRASQDVNTAVAWYQQKPGKAPKLLIYSASFLYSGVPSRFSGSRSGTDFTLTISSLQPEDFATYYCQQHYTTTFGQGTKVEIKRTVAAPSVFIFPPSDEQLKSGTASVVCLLNNFYPREAKVQWKVDNALQSGNSQESVTEQDSKDSTYSLSSTLTLSKADYEKHKVYACEVTHQGLSSPVTKSFNRGEC

SEQ ID NO: 7 - DNA, 65 bp, synthetic construct
  source 1..65: mol_type = other DNA
cctactactgccagcagcactacaccaccccgccgaccttcggtcagggtaccaaagttgaaatc

SEQ ID NO: 8 - DNA, 26 bp, synthetic construct
  source 1..26: mol_type = other DNA
accttcggtcagggtaccaaagttga

SEQ ID NO: 9 - DNA, 25 bp, synthetic construct
  source 1..25: mol_type = other DNA
ggtggtgtagtgctgctggcagtag

SEQ ID NO: 10 - protein, 220 aa, synthetic construct
DVVMTQTPLSLSVTPGEPASISCRSTQSLLDSDGVNPSFDWYVQKPGQSPQLLIHRGFYRASGVPDRFSGSGSGTDFTLRISRVEAEDVGVYYCMQRIEFPLTFGGGTKVEIKRTVAAPSVFIFPPSDEQLKSGTASVVCLLNNFYPREAKVQWKVDNALQSGNSQESVTEQDSKDSTYSLSSTLTLSKADYEKHKLYACEVTHQGLSSPVTKSFNRGEC

SEQ ID NO: 11 - protein, 219 aa, synthetic construct
DVVMTQTPLSLSVTPGEPASISCRSTQSLLDSDGVNPSFDWYVQKPGQSPQLLIHRGFYRASGVPDRFSGSGSGTDFTLRISRVEAEDVGVYYCMQRIEFLTFGGGTKVEIKRTVAAPSVFIFPPSDEQLKSGTASVVCLLNNFYPREAKVQWKVDNALQSGNSQESVTEQDSKDSTYSLSSTLTLSKADYEKHKLYACEVTHQGLSSPVTKSFNRGEC

SEQ ID NO: 12 - protein, 135 aa, synthetic construct
EVQLVESGGGLVQPGGSLRLSCAASGFNIKDTYIHWVRQAPGKGLEWVARIYPTNGYTRYADSVKGRFTISADTSKNTAYLQMNSLRAEDTAVYYCSRWGGDGFYAMDYWGQGTLVTVSSASTKGPSVFPLAPSS

SEQ ID NO: 13 - protein, 265 aa, synthetic construct
MDIQMTQSPSSLSASVGDRVTITCRASQDVNTAVAWYQQKPGKAPKLLIYSASFLYSGVPSRFSGSRSGTDFTLTISSLQPEDFATYYCQQHYTTPPTFGQGTKVEIKRGSGGGGSGGGGSGGGGSKLEVQLVESGGGLVQPGGSLRLSCAASGFNIKDTYIHWVRQAPGKGLEWVARIYPTNGYTRYADSVKGRFTISADTSKNTAYLQMNSLRAEDTAVYYCSRWGGDGFYAMDYWGQGTLVTVSSASTKGPSVFPLAPSSLE

SEQ ID NO: 14 - protein, 263 aa, synthetic construct
MDIQMTQSPSSLSASVGDRVTITCRASQDVNTAVAWYQQKPGKAPKLLIYSASFLYSGVPSRFSGSRSGTDFTLTISSLQPEDFATYYCQQHYTTTFGQGTKVEIKRGSGGGGSGGGGSGGGGSKLEVQLVESGGGLVQPGGSLRLSCAASGFNIKDTYIHWVRQAPGKGLEWVARIYPTNGYTRYADSVKGRFTISADTSKNTAYLQMNSLRAEDTAVYYCSRWGGDGFYAMDYWGQGTLVTVSSASTKGPSVFPLAPSSLE

SEQ ID NO: 15 - protein, 450 aa, synthetic construct
EVQLVESGGGLVQPGGSLRLSCAASGFNIKDTYIHWVRQAPGKGLEWVARIYPTNGYTRYADSVKGRFTISADTSKNTAYLQMNSLRAEDTAVYYCSRWGGDGFYAMDYWGQGTLVTVSSASTKGPSVFPLAPSSKSTSGGTAALGCLVKDYFPEPVTVSWNSGALTSGVHTFPAVLQSSGLYSLSSVVTVPSSSLGTQTYICNVNHKPSNTKVDKKVEPKSCDKTHTCPPCPAPELLGGPSVFLFPPKPKDTLMISRTPEVTCVVVDVSHEDPEVKFNWYVDGVEVHNAKTKPREEQYNSTYRVVSVLTVLHQDWLNGKEYKCKVSNKALPAPIEKTISKAKGQPREPQVYTLPPSREEMTKNQVSLTCLVKGFYPSDIAVEWESNGQPENNYKTTPPVLDSDGSFFLYSKLTVDKSRWQQGNVFSCSVMHEALHNHYTQKSLSLSPGK